European Patent Application EP 4 190 310 A1, published June 7, 2023. Title: Stable Pharmaceutical Formulation. Applicant: CELLTRION, INC. The sequence listing filed with the application follows.

SEQUENCE LISTING (2 sequences)

SEQ ID NO: 1 - DNA, 1377 bp, Artificial Sequence
  Synthetic
atggtcagctactgggacaccggggtcctgctgtgcgcgctgctcagctgtctgcttctcacaggatctagttccggaagtgataccggtagacctttcgtagagatgtacagtgaaatccccgaaattatacacatgactgaaggaagggagctcgtcattccctgccgggttacgtcacctaacatcactgttactttaaaaaagtttccacttgacactttgatccctgatggaaaacgcataatctgggacagtagaaagggcttcatcatatcaaatgcaacgtacaaagaaatagggcttctgacctgtgaagcaacagtcaatgggcatttgtataagacaaactatctcacacatcgacaaaccaatacaatcatagatgtggttctgagtccgtctcatggaattgaactatctgttggagaaaagcttgtcttaaattgtacagcaagaactgaactaaatgtggggattgacttcaactgggaatacccttcttcgaagcatcagcataagaaacttgtaaaccgagacctaaaaacccagtctgggagtgagatgaagaaatttttgagcaccttaactatagatggtgtaacccggagtgaccaaggattgtacacctgtgcagcatccagtgggctgatgaccaagaagaacagcacatttgtcagggtccatgaaaaggacaaaactcacacatgcccaccgtgcccagcacctgaactcctggggggaccgtcagtcttcctcttccccccaaaacccaaggacaccctcatgatctcccggacccctgaggtcacatgcgtggtggtggacgtgagccacgaagaccctgaggtcaagttcaactggtacgtggacggcgtggaggtgcataatgccaagacaaagccgcgggaggagcagtacaacagcacgtaccgtgtggtcagcgtcctcaccgtcctgcaccaggactggctgaatggcaaggagtacaagtgcaaggtctccaacaaagccctcccagcccccatcgagaaaaccatctccaaagccaaagggcagccccgagaaccacaggtgtacaccctgcccccatcccgggatgagctgaccaagaaccaggtcagcctgacctgcctggtcaaaggcttctatcccagcgacatcgccgtggagtgggagagcaatgggcagccggagaacaactacaagaccacgcctcccgtgctggactccgacggctccttcttcctctacagcaagctcaccgtggacaagagcaggtggcagcaggggaacgtcttctcatgctccgtgatgcatgaggctctgcacaaccactacacgcagaagagcctctccctgtctccgggtaaatga

SEQ ID NO: 2 - protein, 458 aa, Artificial Sequence
  Synthetic
MVSYWDTGVLLCALLSCLLLTGSSSGSDTGRPFVEMYSEIPEIIHMTEGRELVIPCRVTSPNITVTLKKFPLDTLIPDGKRIIWDSRKGFIISNATYKEIGLLTCEATVNGHLYKTNYLTHRQTNTIIDVVLSPSHGIELSVGEKLVLNCTARTELNVGIDFNWEYPSSKHQHKKLVNRDLKTQSGSEMKKFLSTLTIDGVTRSDQGLYTCAASSGLMTKKNSTFVRVHEKDKTHTCPPCPAPELLGGPSVFLFPPKPKDTLMISRTPEVTCVVVDVSHEDPEVKFNWYVDGVEVHNAKTKPREEQYNSTYRVVSVLTVLHQDWLNGKEYKCKVSNKALPAPIEKTISKAKGQPREPQVYTLPPSRDELTKNQVSLTCLVKGFYPSDIAVEWESNGQPENNYKTTPPVLDSDGSFFLYSKLTVDKSRWQQGNVFSCSVMHEALHNHYTQKSLSLSPGK